European Patent Application EP 4 365 304 A1, published May 8, 2024. Title: A stem-loop primer and a method for short length RNA detection. Applicant: Universidad Autonoma de Madrid. The sequence listing filed with the application follows.

SEQUENCE LISTING (48 sequences)

SEQ ID NO: 1 - DNA, 50 bp, synthetic construct
  source 1..50: mol_type = other DNA
  stem_loop 1..44
gttggctctggtgcagggtccgacgtattcgcaccagagccaacnnnnnn

SEQ ID NO: 2 - DNA, 22 bp, synthetic construct
  source 1..22: mol_type = other DNA; note = forward primer; note (original language) = cebador directo
ctcgggcgttgnnnnnnnnnnn

SEQ ID NO: 3 - DNA, 17 bp, synthetic construct
  source 1..17: mol_type = other DNA; note = universal reverse primer; note (original language) = cebador reverso universal
cagcctgggacgtggtc

SEQ ID NO: 4 - DNA, 19 bp, synthetic construct
  source 1..19: mol_type = other DNA; note = universal reverse primer; note (original language) = cebador reverso universal
cagcctgggacgtggtctc

SEQ ID NO: 5 - DNA, 19 bp, synthetic construct
  source 1..19: mol_type = other DNA; note = universal reverse primer; note (original language) = cebador reverso universal
tgcagcctgggacgtggtc

SEQ ID NO: 6 - DNA, 22 bp, synthetic construct
  source 1..22: mol_type = other DNA; note = universal probe; note (original language) = sonda universal
caaccgagaccacgcttatgca

SEQ ID NO: 7 - DNA, 25 bp, synthetic construct
  source 1..25: mol_type = other DNA; note = universal probe; note (original language) = sonda universal
caaccgagaccacgcttatgcagcc

SEQ ID NO: 8 - RNA, 22 nt, Homo sapiens
  source 1..22: mol_type = transcribed RNA
  ncRNA 1..22: ncRNA_class = miRNA; note = hsa-miR-146a-5p
tgagaactgaattccatgggtt

SEQ ID NO: 9 - RNA, 24 nt, Homo sapiens
  source 1..24: mol_type = transcribed RNA
  ncRNA 1..24: ncRNA_class = miRNA; note = hsa-miR-155-5p
ttaatgctaatcgtgataggggtt

SEQ ID NO: 10 - RNA, 22 nt, Homo sapiens
  source 1..22: mol_type = transcribed RNA
  ncRNA 1..22: ncRNA_class = miRNA; note = hsa-miR-21-5p
tagcttatcagactgatgttga

SEQ ID NO: 11 - RNA, 22 nt, Homo sapiens
  source 1..22: mol_type = transcribed RNA
  ncRNA 1..22: ncRNA_class = miRNA; note = hsa-miR-194-2-5p
tgtaacagcaactccatgtgga

SEQ ID NO: 12 - RNA, 22 nt, Homo sapiens
  source 1..22: mol_type = transcribed RNA
  ncRNA 1..22: ncRNA_class = miRNA; note = hsa-miR-223-3p
tgtcagtttgtcaaatacccca

SEQ ID NO: 13 - RNA, 21 nt, Homo sapiens
  source 1..21: mol_type = transcribed RNA
  ncRNA 1..21: ncRNA_class = miRNA; note = hsa-miR-192-5p
ctgacctatgaattgacagcc

SEQ ID NO: 14 - RNA, 21 nt, Homo sapiens
  source 1..21: mol_type = transcribed RNA
  ncRNA 1..21: ncRNA_class = miRNA; note = hsa-miR-23a-3p
atcacattgccagggatttcc

SEQ ID NO: 15 - RNA, 23 nt, Homo sapiens
  source 1..23: mol_type = transcribed RNA
  ncRNA 1..23: ncRNA_class = miRNA; note = hsa-miR-200c-3p
taatactgccgggtaatgatgga

SEQ ID NO: 16 - RNA, 22 nt, Homo sapiens
  source 1..22: mol_type = transcribed RNA
  ncRNA 1..22: ncRNA_class = miRNA; note = hsa-miR-22-3p
aagctgccagttgaagaactgt

SEQ ID NO: 17 - RNA, 22 nt, Homo sapiens
  source 1..22: mol_type = transcribed RNA
  ncRNA 1..22: ncRNA_class = miRNA; note = hsa-miR-16-5p
tagcagcacgtaaatattggcg

SEQ ID NO: 18 - RNA, 23 nt, Homo sapiens
  source 1..23: mol_type = transcribed RNA
  ncRNA 1..23: ncRNA_class = miRNA; note = hsa-miR-191-5p
caacggaatcccaaaagcagctg

SEQ ID NO: 19 - RNA, 22 nt, Homo sapiens
  source 1..22: mol_type = transcribed RNA
  ncRNA 1..22: ncRNA_class = miRNA; note = hsa-miR-200a-5p
taacactgtctggtaacgatgt

SEQ ID NO: 20 - RNA, 23 nt, Homo sapiens
  source 1..23: mol_type = transcribed RNA
  ncRNA 1..23: ncRNA_class = miRNA; note = hsa-miR-106a-5p
aaaagtgcttacagtgcaggtag

SEQ ID NO: 21 - DNA, 50 bp, synthetic construct
  source 1..50: mol_type = other DNA; note = hsa-miR-146a-5p stem-loop primer; note (original language) = cebador de bucle en horquilla de hsa-miR-146a-5p
gttggctctggtgcagggtccgacgtattcgcaccagagccaacaaccca

SEQ ID NO: 22 - DNA, 50 bp, synthetic construct
  source 1..50: mol_type = other DNA; note = hsa-miR-155-5pstem-loop primer; note (original language) = cebador de bucle en horquilla de hsa-miR-155-5p
gttggctctggtgcagggtccgacgtattcgcaccagagccaacaacccc

SEQ ID NO: 23 - DNA, 50 bp, synthetic construct
  source 1..50: mol_type = other DNA; note = hsa-miR-21-5p stem-loop primer; note (original language) = cebador de bucle en horquilla de hsa-miR-21-5p
gttggctctggtgcagggtccgacgtattcgcaccagagccaactcaaca

SEQ ID NO: 24 - DNA, 50 bp, synthetic construct
  source 1..50: mol_type = other DNA; note = hsa-miR-194-2-5p stem-loop primer; note (original language) = cebador de bucle en horquilla de hsa-miR-194-2-5p
gttggctctggtgcagggtccgacgtattcgcaccagagccaactccaca

SEQ ID NO: 25 - DNA, 50 bp, synthetic construct
  source 1..50: mol_type = other DNA; note = hsa-miR-223-3p stem-loop primer; note (original language) = cebador de bucle en horquilla de hsa-miR-223-3p
gttggctctggtgcagggtccgacgtattcgcaccagagccaactggggt

SEQ ID NO: 26 - DNA, 50 bp, synthetic construct
  source 1..50: mol_type = other DNA; note = hsa-miR-192-5p stem-loop primer; note (original language) = cebador de bucle en horquilla de hsa-miR-192-5p
gttggctctggtgcagggtccgacgtattcgcaccagagccaacggctgt

SEQ ID NO: 27 - DNA, 50 bp, synthetic construct
  source 1..50: mol_type = other DNA; note = hsa-miR-23a-3p stem-loop primer; note (original language) = cebador de bucle en horquilla de hsa-miR-23a-3p
gttggctctggtgcagggtccgacgtattcgcaccagagccaacggaaat

SEQ ID NO: 28 - DNA, 50 bp, synthetic construct
  source 1..50: mol_type = other DNA; note = hsa-miR-200c-3p stem-loop primer; note (original language) = cebador de bucle en horquilla de hsa-miR-200c-3p
gttggctctggtgcagggtccgacgtattcgcaccagagccaactccatc

SEQ ID NO: 29 - DNA, 50 bp, synthetic construct
  source 1..50: mol_type = other DNA; note = hsa-miR-22-3p stem-loop primer; note (original language) = cebador de bucle en horquilla de hsa-miR-22-3p
gttggctctggtgcagggtccgacgtattcgcaccagagccaacacagtt

SEQ ID NO: 30 - DNA, 50 bp, synthetic construct
  source 1..50: mol_type = other DNA; note = hsa-miR-16-5p stem-loop primer; note (original language) = cebador de bucle en horquilla de hsa-miR-16-5p
gttggctctggtgcagggtccgacgtattcgcaccagagccaaccgccaa

SEQ ID NO: 31 - DNA, 50 bp, synthetic construct
  source 1..50: mol_type = other DNA; note = hsa-miR-191-5p stem-loop primer; note (original language) = cebador de bucle en horquilla de hsa-miR-191-5p
gttggctctggtgcagggtccgacgtattcgcaccagagccaaccagctg

SEQ ID NO: 32 - DNA, 50 bp, synthetic construct
  source 1..50: mol_type = other DNA; note = hsa-miR-200a-5p stem-loop primer; note (original language) = cebador de bucle en horquilla de hsa-miR-200a-5p
gttggctctggtgcagggtccgacgtattcgcaccagagccaacacatcg

SEQ ID NO: 33 - DNA, 50 bp, synthetic construct
  source 1..50: mol_type = other DNA; note = hsa-miR-106a-5p stem-loop primer; note (original language) = cebador de bucle en horquilla de hsa-miR-106a-5p
gttggctctggtgcagggtccgacgtattcgcaccagagccaacctacct

SEQ ID NO: 34 - DNA, 22 bp, synthetic construct
  source 1..22: mol_type = other DNA; note = hsa-miR-146a-5p forward primer; note (original language) = cebador directo de hsa-miR-146a-5p
cgggcgttgtgagaactgaatt

SEQ ID NO: 35 - DNA, 22 bp, synthetic construct
  source 1..22: mol_type = other DNA; note = hsa-miR-155-5p forward primer; note (original language) = cebador directo de hsa-miR-155-5p
cgggcgttgttaatgctaatcg

SEQ ID NO: 36 - DNA, 22 bp, synthetic construct
  source 1..22: mol_type = other DNA; note = hsa-miR-21-5p forward primer; note (original language) = cebador directo de hsa-miR-21-5p
cgggcgttgtagcttatcagac

SEQ ID NO: 37 - DNA, 22 bp, synthetic construct
  source 1..22: mol_type = other DNA; note = hsa-miR-194-2-5p forward primer; note (original language) = cebador directo de hsa-miR-194-2-5p
cgggcgttgtgtaacagcaact

SEQ ID NO: 38 - DNA, 22 bp, synthetic construct
  source 1..22: mol_type = other DNA; note = hsa-miR-223-3p forward primer; note (original language) = cebador directo de hsa-miR-223-3p
cgggcgttgtgtcagtttgtca

SEQ ID NO: 39 - DNA, 22 bp, synthetic construct
  source 1..22: mol_type = other DNA; note = hsa-miR-192-5p forward primer; note (original language) = cebador directo de hsa-miR-192-5p
cgggcgttgctgacctatgaat

SEQ ID NO: 40 - DNA, 22 bp, synthetic construct
  source 1..22: mol_type = other DNA; note = hsa-miR-23a-3p forward primer; note (original language) = cebador directo de hsa-miR-23a-3p
cgggcgttgatcacattgccag

SEQ ID NO: 41 - DNA, 22 bp, synthetic construct
  source 1..22: mol_type = other DNA; note = hsa-miR-200c-3p forward primer; note (original language) = cebador directo de hsa-miR-200c-3p
cgggcgttgtaatactgccggg

SEQ ID NO: 42 - DNA, 22 bp, synthetic construct
  source 1..22: mol_type = other DNA; note = hsa-miR-22-3p forward primer; note (original language) = cebador directo de hsa-miR-22-3p
cgggcgttgaagctgccagttg

SEQ ID NO: 43 - DNA, 22 bp, synthetic construct
  source 1..22: mol_type = other DNA; note = hsa-miR-16-5p forward primer; note (original language) = cebador directo de hsa-miR-16-5p
cgggcgttgtagcagcacgtaa

SEQ ID NO: 44 - DNA, 22 bp, synthetic construct
  source 1..22: mol_type = other DNA; note = hsa-miR-191-5p forward primer; note (original language) = cebador directo de hsa-miR-191-5p
cgggcgttgcaacggaatccca

SEQ ID NO: 45 - DNA, 22 bp, synthetic construct
  source 1..22: mol_type = other DNA; note = hsa-miR-200a-5p forward primer; note (original language) = cebador directo de hsa-miR-200a-5p
cgggcgttgtaacactgtctgg

SEQ ID NO: 46 - DNA, 22 bp, synthetic construct
  source 1..22: mol_type = other DNA; note = hsa-miR-106a-5p forward primer; note (original language) = cebador directo de hsa-miR-106a-5p
cgggcgttgaaaagtgcttaca

SEQ ID NO: 47 - DNA, 11 bp, Araucaria Scopolorum
  source 1..11: mol_type = genomic DNA
ctcgggcgttg

SEQ ID NO: 48 - DNA, 51 bp, synthetic construct
  source 1..51: mol_type = other DNA
  stem_loop 1..44
gttggctctggtgcagggtccgaggtattcgcaccagagccaacnnnnnnn